European Patent Application EP 4 620 964 A1, published September 24, 2025. Title: Peptide Having Activity of Skin Whitening and Uses Thereof. Applicant: CAREGEN CO., LTD. Application KR. The sequence listing filed with the application follows.

SEQUENCE LISTING (9 sequences)

SEQ ID NO: 1 - protein, 4 aa, synthetic construct
ERWW

SEQ ID NO: 2 - DNA, 20 bp, synthetic construct
  source 1..20: mol_type = other DNA
tgctagcagcctctctctcc

SEQ ID NO: 3 - DNA, 20 bp, synthetic construct
  source 1..20: mol_type = other DNA
cttcaaggggaaccagatga

SEQ ID NO: 4 - DNA, 20 bp, synthetic construct
  source 1..20: mol_type = other DNA
ggagccaaaagggtcatcat

SEQ ID NO: 5 - DNA, 20 bp, synthetic construct
  source 1..20: mol_type = other DNA
gtgatggcatggactgtggt

SEQ ID NO: 6 - DNA, 20 bp, synthetic construct
  source 1..20: mol_type = other DNA
gccgtctatttgccacacac

SEQ ID NO: 7 - DNA, 20 bp, synthetic construct
  source 1..20: mol_type = other DNA
gcagtcagcaacttcatggc

SEQ ID NO: 8 - DNA, 20 bp, synthetic construct
  source 1..20: mol_type = other DNA
tgaccaaacgtatccccctg

SEQ ID NO: 9 - DNA, 20 bp, synthetic construct
  source 1..20: mol_type = other DNA
ggtgtctgccgttgaagaga